European Patent Application EP 4 458 960 A1, published November 6, 2024. Title: ENGINEERING BACTERIUM FOR EXPRESSING ASPARTATE DEHYDROGENASE AND METHOD FOR PRODUCING VITAMIN B5 BY FERMENTATION. Applicant: 中国科学院微生物研究所. The sequence listing filed with the application follows.

SEQUENCE LISTING (56 sequences)

SEQ ID NO: 1 - DNA, 384 bp, (Artificial Sequence)
  source 1..384: mol_type = genomic DNA
atgtaccgtacgttaatgagcgcaaaacttcacagagcgagagtgacggaagccaatttgaactacgtcggcagcgtgacaattgatgaagatttgctggatgctgtcggaatgatggcaaatgaaaaagtgcaaattgtgaataataataacggggcccggctggaaacgtacattattcccggtgaaaggggcagcggcgtcgtttgtttaaacggagctgccgcccgccttgtccaggttggagatgtcgtcatcatcgtgtcttatgcgatgatgtctgaagaggaagcaaagacccataagccgaaggttgccgttttgaacgagagaaacgaaatcgaggaaatgctgggtcaggagccagcccgtaccattctgtaa

SEQ ID NO: 2 - DNA, 84 bp, (Artificial Sequence)
  source 1..84: mol_type = genomic DNA
ccaagttcacttaaaaaggagatcaacaatgaaagcaattttcgtactgaaacatcttaatcatgctaaggaggttttctaatg

SEQ ID NO: 3 - DNA, 1800 bp, (Artificial Sequence)
  source 1..1800: mol_type = genomic DNA
cgcggatccttgacaattaatcatccggctcgtataatgtgtggagcacaacatcaatttatcaggatacgttatgaaaccgaccaccatctccttactgcagaagtacaaacaggaaaaaaaacgtttcgcgaccatcaccgcttatgactatagcttcgccaaactctttgctgatgaagggcttaacgtcatgctggtgggcgattcgctgggcatgacggttcaggggcacgactccaccctgccagttaccgttgccgatatcgcctaccacactgccgccgtacgtcgcggcgcaccaaactgcctgctgctggctgacctgccgtttatggcgtatgccacgccggaacaagccttcgaaaacgccgcaacggttatgcgtgccggtgctaacatggtcaaaattgaaggcggtgagtggctggtagaaaccgtacaaatgctgaccgaacgtgccgttcctgtatgtggtcacttaggtttaacaccacagtcagtgaatattttcggtggctacaaagttcaggggcgcggcgatgaagcgggcgatcaactgctcagcgatgcattagccttagaagctgctggggcacagctgctggtgctggaatgcgtgccggttgaactggcaaaacgtattaccgaagcactggcgatcccggttattggcattggcgcaggcaacgtcactgacgggcagatcctcgtgatgcacgacgcctttggtattaccggcggtcacattcctaaattcgctaaaaatttcctcgccgaaacgggcgacatccgcgcggctgtgcggcagtatatggctgaagtggagtccggcgtttatccgggcgaagaacacagtttccattaaggagtcacgttgtgttaattatcgaaaccctgccgctgctgcgtcagcaaattcgccgcctgcgtatggaaggcaagcgcgtggcgctggtgcctaccatgggtaacctgcacgatggccatatgaagctggtcgacgaagccaaagcccgcgccgatgtggtcgtcgtcagtattttcgttaacccgatgcagttcgaccgcccggaagatctggctcgttatccacggaccttgcaggaggactgcgagaagctaaacaaacgtaaagtggatttagttttcgccccttcggtaaaagagatctacccgaacggtactgaaacccacacttacgttgacgttcctggcctttcgaccatgctggaaggtgccagccgtccgggacattttcgcggcgtttcgactattgtcagcaagctgttcaacctggtccagccggacatcgcctgcttcggtgaaaaagattttcagcaactggcgctgatccgcaaaatggttgccgatatgggcttcgatattgagattgtcggtgtgccaattatgcgcgccaaagacggtctggcgctaagttcccgtaacggttatctgacggcggaacaacgcaaaattgcgcctggtctgtacaaagttttaagttcgattgctgacaaattgcaggctggggaacgggatctcgatgaaattattaccattgcggggcaagaactgaatgaaaaaggcttccgcgccgatgatattcagattcgcgatgccgacacattgctggaagtttctgaaaccagcaaacgggcagtaattctggtagccgcctggcttggcgatgctcgcctgatcgacaacaaaatggtcgagctggcgtaatacttaactggcgctacggctgatggcgccagttattaatttaccccacgtcatctgtcataacacagg

SEQ ID NO: 4 - DNA, 1044 bp, (Artificial Sequence)
  source 1..1044: mol_type = genomic DNA
acatgcatgcttgacagctagctcagtcctaggtataatgctagcgttgcgggtgaggaggaacaatgaaaattaccgtattgggatgcggtgccttagggcaattatggcttacagcactttgcaaacagggtcatgaagttcagggctggctgcgcgtaccgcaaccttattgtagcgtgaatctggttgagacagatggttcgatatttaacgaatcgctgaccgccaacgatcccgattttctcgccaccagcgatctgctcctggtgacgctgaaagcatggcaggtttccgatgccgtcaaaagcctcgcgtccacactgcctgtaactacgccaatactgttaattcacaacggcatgggcaccatcgaagagttgcaaaacattcagcagccattactgatgggcaccaccacccatgcagcccgccgcgacggcaatgtcattattcatgtggcaaacggtatcacgcatattggcccggcacggcaacaggacggggattacagttatctggcggatattttgcaaaccgtgttgcctgacgttgcctggcataacaatattcgcgccgagctgtggcgcaagctggcagtcaactgcgtgattaatccactgactgccatctggaattgcccgaacggtgaattacgtcatcatccgcaagaaattatgcagatatgcgaagaagtcgcggcggtgatcgaacgcgaagggcatcatacttcagcagaagatttgcgtgattacgtgatgcaggtgattgatgccacagcggaaaatatctcgtcgatgttgcaggatatccgcgcgctgcgccacactgaaatcgactatatcaatggttttctcttacgccgcgcccgcgcgcatgggattgccgtaccggaaaacacccgcctgtttgaaatggtaaaaagaaaggagagtgaatatgagcgcatcggcactggtttgcctcgcccctggtagtgaagagactaattttcgaaaaaagacgctgaaaagcgtcttttttcgttttgggatctaaatcgag

SEQ ID NO: 5 - DNA, 1261 bp, (Artificial Sequence)
  source 1..1261: mol_type = genomic DNA
cggactggaagaagatctgtttgtctctgcgcgtccgaatattgaactgctgccggaaggccagtttaaataccacgtcgattttgagcatctgcatattggcgaagaaaccgggatgatttgcgtctcccggccgacgaatccaacaggcaatgtgattactgacgaagagttgctgaagcttgacgcgctggcgaatcaacacggcattccgctggtgattgataacgcttatggcgtcccgttcccgggtatcatcttcagtgaagcgcgcccgctatggaatccgaatatcgtgctgtgcatgagtctcaattccgacgtctaagaaaccattattatcatgacattaacctataaaaataggcgtatcacgaggccctttcgtcttcacctcgagtccctatcagtgatagagattgacatccctatcagtgatagagatactgagcacatcagcaggacgcactgaccgggcccaagttcacttaaaaaggagatcaacaatgaaagcaattttcgtactgaaacatcttaatcatgctaaggaggttttctaatgtaccgtacgttaatgagcgcaaaacttcacagagcgagagtgacggaagccaatttgaactacgtcggcagcgtgacaattgatgaagatttgctggatgctgtcggaatgatggcaaatgaaaaagtgcaaattgtgaataataataacggggcccggctggaaacgtacattattcccggtgaaaggggcagcggcgtcgtttgtttaaacggagctgccgcccgccttgtccaggttggagatgtcgtcatcatcgtgtcttatgcgatgatgtctgaagaggaagcaaagacccataagccgaaggttgccgttttgaacgagagaaacgaaatcgaggaaatgctgggtcaggagccagcccgtaccattctgtaaaagcctagcataaccccttggggcctctaaacgggtcttgaggggttttttgcatcaccaatatgaacggcattatcagcctggcacctggcggtattggtccggcgatgatgtgtgaaatgattaagcgtaacgatctgctgcgcctgtctgaaacagtcatcaaaccgttttactaccagcgtgttcaggaaactatcgccatcattcgccgctatttaccggaaaatcgctgcctgattcataaaccggaaggagccattttcctctggctatggtttaaggatttgcccattacgaccaagcagctctatcagc

SEQ ID NO: 6 - DNA, 2629 bp, (Artificial Sequence)
  source 1..2629: mol_type = genomic DNA
ggcagaaaatcagccagttccgcgcccgccatcccgcaattggcgcgggcaaacaaacgacacttttgctgaagcagggctacggctttgttcgtgagcatggcgacgataaagtgctggtcgtctgggcagggcaacagtaacttttccggcttcccgttcgtcagtacctcgggaagccgccaaccaggataaaatgtcagccctaatcagcgttgcaggataaagcaccgctcactcttcaacagaccgatttgcaccccagcaaatgtagcgttattgttaccttccttgctacagagttcttgacaattaatcatccggctcgtataatgtgtggacaagattcaggacggggaactaactatgaatggcgcacagtgggtggtacatgcgttgcgggcacagggtgtgaacaccgttttcggttatccgggtggcgcaattatgccggtttacgatgcattgtatgacggcggcgtggagcacttgctatgccgacatgagcagggtgcggcaatggcggctatcggttatgctcgtgctaccggcaaaactggcgtatgtatcgccacgtctggtccgggcgcaaccaacctgataaccgggcttgcggacgcactgttagattccatccctgttgttgccatcaccggtcaagtgtccgcaccgtttatcggcactgacgcatttcaggaagtggatgtcctgggattgtcgttagcctgtaccaagcacagctttctggtgcagtcgctggaagagttgccgcgcatcatggctgaagcattcgacgttgcctgctcaggtcgtcctggtccggttctggtcgatatcccaaaagatatccagttagccagcggtgacctggaaccgtggttcaccaccgttgaaaacgaagtgactttcccacatgccgaagttgagcaagcgcgccagatgctggcaaaagcgcaaaaaccgatgctgtacgttggcggtggcgtgggtatggcgcaggcagttccggctttgcgtgaatttctcgctgccacaaaaatgcctgccacctgtacgctgaaagggctgggcgcagtagaagcagattatccgtactatctgggcatgctgggaatgcatggcaccaaagcggcgaacttcgcggtgcaggagtgcgacttgctgatcgccgtgggtgcacgttttgatgaccgggtgaccggcaaactgaacaccttcgcaccacacgccagtgttatccatatggatatcgacccggcagaaatgaacaagctgcgtcaggcacatgtggcattacaaggtgatttaaatgctctgttaccagcattacagcagccgttaaatatcaatgactggcagctacactgcgcgcagctgcgtgatgaacatgcctggcgttacgaccatcccggtgacgctatctacgcgccgttgttgttaaaacaactgtcagatcgtaaacctgcggattgcgtcgtgaccacagatgtggggcagcaccagatgtgggctgcgcagcacatcgcccacactcgcccggaaaatttcatcacctccagcggcttaggcaccatgggttttggtttaccggcggcggttggcgcgcaagtcgcgcgaccaaacgataccgtcgtctgtatctccggtgacggctctttcatgatgaatgtgcaagagctgggcaccgtaaaacgcaagcagttaccgttgaaaatcgtcttactcgataaccaacggttagggatggttcgacaatggcagcaactgtttttccaggaacgatatagcgaaaccacccttaccgataaccccgatttcctcatgttagccagcgccttcggcatccctggccaacacatcacccgtaaagaccaggttgaagcggcactcgacaccatgctgaacagtgatgggccatacctgcttcatgtctcaatcgacgaacttgagaacgtctggccgctggtgccgcctggtgccagtaattcagaaatgttggagaaattatcatgatgcaacatcaggtcaatgtatcggctcgcttcaatccagaaaccttagaacgtgttttacgcgtggtgcgtcatcgtggtttccacgtctgctcaatgaatatggccgccgccagcgatgcacaaaatataaatatcgaattgaccgttgccagcccacggtcggtcgacttactgtttagtcagttaaataaactggtggacgtcgcacacgttgccatctgccagagcacaaccacatcacaacaaatccgcgcctgagcgcaaaaggaatataccagaaaagagacgcttttagagcgtcttttttcgttttggagctactcacactgcttgccggaatgctgcgcgagaagttgggttgggatatcgaaccacagaatattgcactaacaaacggcagccagagcgcgtttttctacttatttaacctgtttgccggacgccgtgccgatggtcgggtcaaaaaagtgctgttcccgcttgcaccggaatacattggctatgctgacgccggactggaagaagatctgtttgtctctgcgcgtccgaatattgaactgctgccggaaggccagtttaaataccacgtcgattttgagcatctgcatattggc

SEQ ID NO: 7 - DNA, 1535 bp, (Artificial Sequence)
  source 1..1535: mol_type = genomic DNA
gttgcgtgttctgcttcatcgcgctgatgggcgcaagctccttcgagctggcaggtaccttcatcgtcagcctgattatcctgatgttctacgctcgcaaaatgcacgagcgccagagccactcaatggataaccacaccgcgtctaacgcacattaattaaaagtattttccgaggctcctcctttcattttgtcccatgtgttgggagcaaaacattaacaccaactggcaaaattttgtcctaaacttgatctcgacgaaatggctgcacctaaatcgtgatgaaaatcacatttttatcgtaattgccctttaaaattcggggcgccgaccccatgtggtctcaagcccaaaggaagagtgaggcgagtcagtcgcgtaatgcttaggcacaggattgatttgtcgcaatgattgacacgattccgcttgacgctgcgtaaggtttttgtaattttacaggcaaccttttattcaccatcttaatcatgctaaggaggttttctaatgaatattgctgtgattggctgcggtgcgattggcgccagcgtgctcgaactgctcaagggccatgccgcggtgcaggtgggctgggtgcttgtgcccgaagtgacggacgccgtgcgcgccaccctggcccggcatgcgccccaggcgcgcgcactgcctgcgctgacgactgaagaccggcccgaccttatcgtcgaatgcgcaggccataccgccatcgaagagcatgtgctgcccgccctgcggcgcggcattcctgccgtcgtggcctccatcggcgcactcagcgcccccggcatggccgaggccgttcaggccgcggccgaggccggaggcacccaggtgcaattgctgtcgggcgccatcggcggcgtggatgcgctggccgcagcccgcatcggcggcctggacgaagtggtctacaccggccgcaagccgcccctggcctggaccggcacgcccgcagaacagcgctgcgacctcgccagcctcaaggaagccttctgcatcttcgaaggcagcgcacgcgaggccgcccagctctaccccaagaacgccaacgtggccgccaccctgtcgctggccggcatgggcctggaccgcaccacggtgcgcctgtacgccgacccggccgtggacgaaaacgtgcaccatgtggccgcgcgcggcgccttcggttccatggaattgaccatgcgcggcaagccgctggaggccaaccccaagacctcggccctcaccgtctacagcgtggtgcgcgccgtgctcaaccaggccacggccatcgccatctaagccgcaccttttcgaaaaaagacgctgaaaagcgtcttttttcgttttggtccagctgtgcgaagaaattagcaaaatgaacgagaacctgccgttgtacgcgttcgctaatacgtattccactctcgatgtaagcctgaatgacctgcgtttacagattagcttctttgaatatgcgctgggtgctgctgaagatattgctaataagatcaagcagaccactgacga

SEQ ID NO: 8 - DNA, 2166 bp, (Artificial Sequence)
  source 1..2166: mol_type = genomic DNA
gttgcgtgttctgcttcatcgcgctgatgggcgcaagctccttcgagctggcaggtaccttcatcgtcagcctgattatcctgatgttctacgctcgcaaaatgcacgagcgccagagccactcaatggataaccacaccgcgtctaacgcacattaattaaaagtattttccgaggctcctcctttcattttgtcccatgtgttgggagcaaaacattaacaccaactggcaaaattttgtcctaaacttgatctcgacgaaatggctgcacctaaatcgtgatgaaaatcacatttttatcgtaattgccctttaaaattcggggcgccgaccccatgtggtctcaagcccaaaggaagagtgaggcgagtcagtcgcgtaatgcttaggcacaggattgatttgtcgcaatgattgacacgattccgcttgacgctgcgtaaggtttttgtaattttacaggcaaccttttattcactataccttccagagcaatctcacgtcttgcaaaaacagcctgcgttttcatcagtaatagttggaattttgtaaatctcccgttaccctgatagcggacttcccttctgtaaccataatggaacctcgtcatgtttgagaacattaccgccgctcctgccgacccgattctgggcctggccgatctgtttcgtgccgatgaacgtcccggcaaaattaacctcgggattggtgtctataaagatgagacgggcaaaaccccggtactgaccagcgtgaaaaaggctgaacagtatctgctcgaaaatgaaaccaccaaaaattacctcggcattgacggcatccctgaatttggtcgctgcactcaggaactgctgtttggtaaaggtagcgccctgatcaatgacaaacgtgctcgcacggcacagactccggggggcactggcgcactacgcgtggctgccgatttcctggcaaaaaataccagcgttaagcgtgtgtgggtgagcaacccaagctggccgaaccataagagcgtctttaactctgcaggtctggaagttcgtgaatacgcttattatgatgcggaaaatcacactcttgacttcgatgcactgattaacagcctgaatgaagctcaggctggcgacgtagtgctgttccatggctgctgccataacccaaccggtatcgaccctacgctggaacaatggcaaacactggcacaactctccgttgagaaaggctggttaccgctgtttgacttcgcttaccagggttttgcccgtggtctggaagaagatgctgaaggactgcgcgctttcgcggctatgcataaagagctgattgttgccagttcctactctaaaaactttggcctgtacaacgagcgtgttggcgcttgtactctggttgctgccgacagtgaaaccgttgatcgcgcattcagccaaatgaaagcggcgattcgcgctaactactctaacccaccagcacacggcgcttctgttgttgccaccatcctgagcaacgatgcgttacgtgcgatttgggaacaagagctgactgatatgcgccagcgtattcagcgtatgcgtcagttgttcgtcaatacgctgcaggaaaaaggcgcaaaccgcgacttcagctttatcatcaaacagaacggcatgttctccttcagtggcctgacaaaagaacaagtgctgcgtctgcgcgaagagtttggcgtatatgcggttgcttctggtcgcgtaaatgtggccgggatgacaccagataacatggctccgctgtgcgaagcgattgtggcagtgctgtaagcattaaaaacaatgaagcccgctgaaaagcgggctgagactgatgacaaacgcaacattgcctgatgcgctacgcttatcaggcctacgcgtcccctgcaatattttgaatttgcacgattttgtaggccggataaggcgctcgtgccgcatccggcataaacaaagcgcactttgccagaaatccaggagctgtgcgaagaaattagcaaaatgaacgagaacctgccgttgtacgcgttcgctaatacgtattccactctcgatgtaagcctgaatgacctgcgtttacagattagcttctttgaatatgcgctgggtgctgctgaagatattgctaataagatcaagcagaccactgacga

SEQ ID NO: 9 - DNA, 2178 bp, (Artificial Sequence)
  source 1..2178: mol_type = genomic DNA
gttgcgtgttctgcttcatcgcgctgatgggcgcaagctccttcgagctggcaggtaccttcatcgtcagcctgattatcctgatgttctacgctcgcaaaatgcacgagcgccagagccactcaatggataaccacaccgcgtctaacgcacattaattaaaagtattttccgaggctcctcctttcattttgtcccatgtgttgggagcaaaacattaacaccaactggcaaaattttgtcctaaacttgatctcgacgaaatggctgcacctaaatcgtgatgaaaatcacatttttatcgtaattgccctttaaaattcggggcgccgaccccatgtggtctcaagcccaaaggaagagtgaggcgagtcagtcgcgtaatgcttaggcacaggattgatttgtcgcaatgattgacacgattccgcttgacgctgcgtaaggtttttgtaattttacaggcaaccttttattcacgcagcttgaaaaagaaggttcacatgtcaaacaacattcgtatcgaagaagatctgttgggtaccagggaagttccagctgatgcctactatggtgttcacactctgagagcgattgaaaacttctatatcagcaacaacaaaatcagtgatattcctgaatttgttcgcggtatggtaatggttaaaaaagccgcagctatggcaaacaaagagctgcaaaccattcctaaaagtgtagcgaatgccatcattgccgcatgtgatgaagtcctgaacaacggaaaatgcatggatcagttcccggtagacgtctaccagggcggcgcaggtacttccgtaaacatgaacaccaacgaagtgctggccaatatcggtctggaactgatgggtcaccaaaaaggtgaatatcagtacctgaacccgaacgaccatgttaacaaatgtcagtccactaacgacgcctacccgaccggtttccgtatcgcagtttactcttccctgattaagctggtagatgcgattaaccaactgcgtgaaggctttgaacgtaaagctgtcgaattccaggacatcctgaaaatgggtcgtacccagctgcaggacgcagtaccgatgaccctcggtcaggaattccgcgctttcagcatcctgctgaaagaagaagtgaaaaacatccaacgtaccgctgaactgctgctggaagttaaccttggtgcaacagcaatcggtactggtctgaacacgccgaaagagtactctccgctggcagtgaaaaaactggctgaagttactggcttcccatgcgtaccggctgaagacctgatcgaagcgacctctgactgcggcgcttatgttatggttcacggcgcgctgaaacgcctggctgtgaagatgtccaaaatctgtaacgacctgcgcttgctctcttcaggcccacgtgccggcctgaacgagatcaacctgccggaactgcaggcgggctcttccatcatgccagctaaagtaaacccggttgttccggaagtggttaaccaggtatgcttcaaagtcatcggtaacgacaccactgttaccatggcagcagaagcaggtcagctgcagttgaacgttatggagccggtcattggccaggccatgttcgaatccgttcacattctgaccaacgcttgctacaacctgctggaaaaatgcattaacggcatcactgctaacaaagaagtgtgcgaaggttacgtttacaactctatcggtatcgttacttacctgaacccgttcatcggtcaccacaacggtgacatcgtgggtaaaatctgtgccgaaaccggtaagagtgtacgtgaagtcgttctggaacgcggtctgttgactgaagcggaacttgacgatattttctccgtacagaatctgatgcacccggcttacaaagcaaaacgctatactgatgaaagcgaacagtaatcgtacagggtagtacaaataaaaaaggcacgtcagatgacgtgccttttttcttgtgagcagagctgtgcgaagaaattagcaaaatgaacgagaacctgccgttgtacgcgttcgctaatacgtattccactctcgatgtaagcctgaatgacctgcgtttacagattagcttctttgaatatgcgctgggtgctgctgaagatattgctaataagatcaagcagaccactgacga

SEQ ID NO: 10 - DNA, 63 bp, (Artificial Sequence)
  source 1..63: mol_type = genomic DNA
cgcggatcccaattaatcatccggctcgtataatgtgtggagcacaacatcaatttatcagga

SEQ ID NO: 11 - DNA, 30 bp, (Artificial Sequence)
  source 1..30: mol_type = genomic DNA
acatgcatgccctgtgttatgacagatgac

SEQ ID NO: 12 - DNA, 65 bp, (Artificial Sequence)
  source 1..65: mol_type = genomic DNA
acatgcatgcttgacagctagctcagtcctaggtataatgctagcgttgcgggtgaggaggaaca

SEQ ID NO: 13 - DNA, 90 bp, (Artificial Sequence)
  source 1..90: mol_type = genomic DNA
ctcgatttagatcccaaaacgaaaaaagacgcgcttttcagcgtcttttttcgaaaattagtctcttcactaccagggatgactatcgag

SEQ ID NO: 14 - DNA, 30 bp, (Artificial Sequence)
  source 1..30: mol_type = genomic DNA
tgggtctaccgttttagagctagaaatagc

SEQ ID NO: 15 - DNA, 29 bp, (Artificial Sequence)
  source 1..29: mol_type = genomic DNA
gcttggaaaggactagtattatacctagg

SEQ ID NO: 16 - DNA, 19 bp, (Artificial Sequence)
  source 1..19: mol_type = genomic DNA
cggactggaagaagatctg

SEQ ID NO: 17 - DNA, 39 bp, (Artificial Sequence)
  source 1..39: mol_type = genomic DNA
tttcttagacgtcggaattgagactcatgcacagcacga

SEQ ID NO: 18 - DNA, 40 bp, (Artificial Sequence)
  source 1..40: mol_type = genomic DNA
tcgtgctgtgcatgagtctcaattccgacgtctaagaaac

SEQ ID NO: 19 - DNA, 44 bp, (Artificial Sequence)
  source 1..44: mol_type = genomic DNA
gatctcctttttaagtgaacttggggtcagtgcgtcctgctgat

SEQ ID NO: 20 - DNA, 44 bp, (Artificial Sequence)
  source 1..44: mol_type = genomic DNA
atcagcaggacgcactgaccccaagttcacttaaaaaggagatc

SEQ ID NO: 21 - DNA, 39 bp, (Artificial Sequence)
  source 1..39: mol_type = genomic DNA
tgccgttcatattggtgatgcaaaaaacccctcaagacc

SEQ ID NO: 22 - DNA, 39 bp, (Artificial Sequence)
  source 1..39: mol_type = genomic DNA
ggtcttgaggggttttttgcatcaccaatatgaacggca

SEQ ID NO: 23 - DNA, 19 bp, (Artificial Sequence)
  source 1..19: mol_type = genomic DNA
gctgatagagctgcttggt

SEQ ID NO: 24 - DNA, 20 bp, (Artificial Sequence)
  source 1..20: mol_type = genomic DNA
ggagctactcacactgcttg

SEQ ID NO: 25 - DNA, 20 bp, (Artificial Sequence)
  source 1..20: mol_type = genomic DNA
cgcatacattgatgcgtatg

SEQ ID NO: 26 - DNA, 30 bp, (Artificial Sequence)
  source 1..30: mol_type = genomic DNA
acggtccacagttttagagctagaaatagc

SEQ ID NO: 27 - DNA, 29 bp, (Artificial Sequence)
  source 1..29: mol_type = genomic DNA
cgtagttacagactagtattatacctagg

SEQ ID NO: 28 - DNA, 20 bp, (Artificial Sequence)
  source 1..20: mol_type = genomic DNA
ggcagaaaatcagccagttc

SEQ ID NO: 29 - DNA, 56 bp, (Artificial Sequence)
  source 1..56: mol_type = genomic DNA
tccacacattatacgagccggatgattaattgtcaagaactctgtagcaaggaagg

SEQ ID NO: 30 - DNA, 56 bp, (Artificial Sequence)
  source 1..56: mol_type = genomic DNA
ttgacaattaatcatccggctcgtataatgtgtggacaagattcaggacggggaac

SEQ ID NO: 31 - DNA, 55 bp, (Artificial Sequence)
  source 1..55: mol_type = genomic DNA
cgaaaaaagacgctctaaaagcgtctcttttctggtatattccttttgcgctcag

SEQ ID NO: 32 - DNA, 58 bp, (Artificial Sequence)
  source 1..58: mol_type = genomic DNA
cagaaaagagacgcttttagagcgtcttttttcgttttggagctactcacactgcttg

SEQ ID NO: 33 - DNA, 38 bp, (Artificial Sequence)
  source 1..38: mol_type = genomic DNA
gccaatatgcagatgctcatgagcatctgcatattggc

SEQ ID NO: 34 - DNA, 19 bp, (Artificial Sequence)
  source 1..19: mol_type = genomic DNA
cacgttcggatatgaactg

SEQ ID NO: 35 - DNA, 19 bp, (Artificial Sequence)
  source 1..19: mol_type = genomic DNA
cgtcaagcttcagcaactc

SEQ ID NO: 36 - DNA, 30 bp, (Artificial Sequence)
  source 1..30: mol_type = genomic DNA
tcatatctccgttttagagctagaaatagc

SEQ ID NO: 37 - DNA, 29 bp, (Artificial Sequence)
  source 1..29: mol_type = genomic DNA
ctatgaacgtgactagtattatacctagg

SEQ ID NO: 38 - DNA, 20 bp, (Artificial Sequence)
  source 1..20: mol_type = genomic DNA
gttgcgtgttctgcttcatc

SEQ ID NO: 39 - DNA, 39 bp, (Artificial Sequence)
  source 1..39: mol_type = genomic DNA
ccagttggtgttaatgttttgctcccaacacatgggaca

SEQ ID NO: 40 - DNA, 39 bp, (Artificial Sequence)
  source 1..39: mol_type = genomic DNA
tgtcccatgtgttgggagcaaaacattaacaccaactgg

SEQ ID NO: 41 - DNA, 41 bp, (Artificial Sequence)
  source 1..41: mol_type = genomic DNA
ctccttagcatgattaagatggtgaataaaaggttgcctgt

SEQ ID NO: 42 - DNA, 41 bp, (Artificial Sequence)
  source 1..41: mol_type = genomic DNA
acaggcaaccttttattcaccatcttaatcatgctaaggag

SEQ ID NO: 43 - DNA, 41 bp, (Artificial Sequence)
  source 1..41: mol_type = genomic DNA
gctaatttcttcgcacagctggaccaaaacgaaaaaagacg

SEQ ID NO: 44 - DNA, 41 bp, (Artificial Sequence)
  source 1..41: mol_type = genomic DNA
cgtcttttttcgttttggtccagctgtgcgaagaaattagc

SEQ ID NO: 45 - DNA, 19 bp, (Artificial Sequence)
  source 1..19: mol_type = genomic DNA
tcgtcagtggtctgcttga

SEQ ID NO: 46 - DNA, 20 bp, (Artificial Sequence)
  source 1..20: mol_type = genomic DNA
ctactcttgcgttgacctga

SEQ ID NO: 47 - DNA, 20 bp, (Artificial Sequence)
  source 1..20: mol_type = genomic DNA
gtgaccaggagtacagaaag

SEQ ID NO: 48 - DNA, 41 bp, (Artificial Sequence)
  source 1..41: mol_type = genomic DNA
gagattgctctggaaggtatagtgaataaaaggttgcctgt

SEQ ID NO: 49 - DNA, 41 bp, (Artificial Sequence)
  source 1..41: mol_type = genomic DNA
acaggcaaccttttattcactataccttccagagcaatctc

SEQ ID NO: 50 - DNA, 40 bp, (Artificial Sequence)
  source 1..40: mol_type = genomic DNA
gctaatttcttcgcacagctcctggatttctggcaaagtg

SEQ ID NO: 51 - DNA, 40 bp, (Artificial Sequence)
  source 1..40: mol_type = genomic DNA
cactttgccagaaatccaggagctgtgcgaagaaattagc

SEQ ID NO: 52 - DNA, 41 bp, (Artificial Sequence)
  source 1..41: mol_type = genomic DNA
gaaccttctttttcaagctgcgtgaataaaaggttgcctgt

SEQ ID NO: 53 - DNA, 41 bp, (Artificial Sequence)
  source 1..41: mol_type = genomic DNA
acaggcaaccttttattcacgcagcttgaaaaagaaggttc

SEQ ID NO: 54 - DNA, 40 bp, (Artificial Sequence)
  source 1..40: mol_type = genomic DNA
gctaatttcttcgcacagctctgctcacaagaaaaaaggc

SEQ ID NO: 55 - DNA, 40 bp, (Artificial Sequence)
  source 1..40: mol_type = genomic DNA
gccttttttcttgtgagcagagctgtgcgaagaaattagc

SEQ ID NO: 56 - DNA, 798 bp, (Artificial Sequence)
  source 1..798: mol_type = genomic DNA
atgaatattgctgtgattggctgcggtgcgattggcgccagcgtgctcgaactgctcaagggccatgccgcggtgcaggtgggctgggtgcttgtgcccgaagtgacggacgccgtgcgcgccaccctggcccggcatgcgccccaggcgcgcgcactgcctgcgctgacgactgaagaccggcccgaccttatcgtcgaatgcgcaggccataccgccatcgaagagcatgtgctgcccgccctgcggcgcggcattcctgccgtcgtggcctccatcggcgcactcagcgcccccggcatggccgaggccgttcaggccgcggccgaggccggaggcacccaggtgcaattgctgtcgggcgccatcggcggcgtggatgcgctggccgcagcccgcatcggcggcctggacgaagtggtctacaccggccgcaagccgcccctggcctggaccggcacgcccgcagaacagcgctgcgacctcgccagcctcaaggaagccttctgcatcttcgaaggcagcgcacgcgaggccgcccagctctaccccaagaacgccaacgtggccgccaccctgtcgctggccggcatgggcctggaccgcaccacggtgcgcctgtacgccgacccggccgtggacgaaaacgtgcaccatgtggccgcgcgcggcgccttcggttccatggaattgaccatgcgcggcaagccgctggaggccaaccccaagacctcggccctcaccgtctacagcgtggtgcgcgccgtgctcaaccaggccacggccatcgccatctaa